European Patent Application EP 4 230 653 A1, published August 23, 2023. Title: ANTI-HER3 ANTIBODY AND ANTI-HER3 ANTIBODY-DRUG CONJUGATE AND MEDICAL USE THEREOF. Applicant: Jiangsu Hengrui Pharmaceuticals Co., Ltd. Shanghai Hengrui Pharmaceutical Co., Ltd. The sequence listing filed with the application follows.

SEQUENCE LISTING (28 sequences)

SEQ ID NO: 1 - protein, 624 aa, Artificial Sequence
  PEPTIDE: Amino acid sequence of HuMan ErbB3
SEVGNSQAVCPGTLNGLSVTGDAENQYQTLYKLYERCEVVMGNLEIVLTGHNADLSFLQWIREVTGYVLVAMNEFSTLPLPNLRVVRGTQVYDGKFAIFVMLNYNTNSSHALRQLRLTQLTEILSGGVYIEKNDKLCHMDTIDWRDIVRDRDAEIVVKDNGRSCPPCHEVCKGRCWGPGSEDCQTLTKTICAPQCNGHCFGPNPNQCCHDECAGGCSGPQDTDCFACRHFNDSGACVPRCPQPLVYNKLTFQLEPNPHTKYQYGGVCVASCPHNFVVDQTSCVRACPPDKMEVDKNGLKMCEPCGGLCPKACEGTGSGSRFQTVDSSNIDGFVNCTKILGNLDFLITGLNGDPWHKIPALDPEKLNVFRTVREITGYLNIQSWPPHMHNFSVFSNLTTIGGRSLYNRGFSLLIMKNLNVTSLGFRSLKEISAGRIYISANRQLCYHHSLNWTKVLRGPTEERLDIKHNRPRRDCVAEGKVCDPLCSSGGCWGPGPGQCLSCRNYSRGGVCVTHCNFLNGEPREFAHEAECFSCHPECQPMEGTATCNGSGSDTCAQCAHFRDGPHCVSSCPHGVLGAKGPIYKYPDVQNECRPCHENCTQGCKGPELQDCLGQTLVLIGKTHLT

SEQ ID NO: 2 - DNA, 1872 bp, Artificial Sequence
  gene: Nucleotide sequence of HuMan ErbB3
agcgaagtcggcaacagccaagccgtctgtcccggcacactcaatggactgtccgtgactggcgacgccgagaaccaataccagacactctacaagctctacgagaggtgcgaggtggtcatgggaaatctggagatcgtgctgactggccataacgccgatctgtcctttctgcagtggattagggaagtgactggctacgtgctggtcgccatgaatgagttttccactctgccactgccaaatctgagagtggtgaggggcactcaagtgtacgacggcaagttcgccattttcgtcatgctcaactacaacacaaactccagccacgccctcagacagctgaggctcactcagctgacagaaattctgtccggcggcgtctatatcgagaaaaacgataaactgtgccacatggacacaatcgattggagggacatcgtgagggatagggatgccgagatcgtggtcaaggataacggaaggagctgtcctccttgtcatgaggtctgcaagggaaggtgttggggacccggctccgaagactgccagacactgactaagactatctgcgcccctcagtgcaatggacactgcttcggcccaaatccaaaccagtgctgccacgacgaatgtgccggcggatgcagcggaccacaagatacagactgcttcgcttgtagacacttcaatgactccggcgcttgtgtgcctaggtgtccacagccactcgtgtacaacaagctcacttttcagctcgagcctaaccctcacactaagtaccaatacggcggagtctgcgtcgccagctgtcctcacaacttcgtggtggatcagacaagctgcgtgagagcttgccctccagataaaatggaggtggacaagaacggactgaagatgtgtgagccttgcggcggactgtgtcctaaagcttgcgagggcactggctccggatctaggttccagactgtcgactccagcaacatcgacggctttgtgaactgcactaagattctgggcaatctggactttctgatcactggcctcaacggcgatccttggcacaagatcccagctctggacccagaaaagctgaatgtgtttaggacagtgagggagattactggctacctcaacatccagagctggcctccacacatgcacaacttcagcgtgttctccaatctgactacaatcggcggcagatccctctataataggggcttctctctgctcatcatgaagaatctgaacgtcacttctctgggcttcagatctctgaaggagatctccgccggaaggatttacatctccgccaataggcagctctgttaccaccacagcctcaactggactaaggtgctgaggggacctactgaggaaaggctggacattaaacacaataggccaagaagggattgcgtcgctgagggcaaagtgtgtgatcctctgtgtagctccggaggatgttggggacccggccccggccagtgtctgagctgtaggaattattctaggggcggcgtgtgtgtgacacactgcaactttctgaacggcgaacctagggaattcgcccatgaagccgagtgcttcagctgccacccagagtgtcagcctatggagggcacagctacatgcaatggcagcggatccgacacatgtgctcagtgtgcccactttagggatggacctcattgcgtcagcagctgtccacacggcgtgctgggagccaagggccctatctacaagtacccagatgtgcagaacgagtgtaggccttgccacgagaattgcacacaaggctgcaagggcccagagctgcaagattgcctcggccagactctggtgctcatcggcaagactcatctcact

SEQ ID NO: 3 - protein, 447 aa, Artificial Sequence
  CHAIN: Heavy chain of U3
QVQLQQWGAGLLKPSETLSLTCAVYGGSFSGYYWSWIRQPPGKGLEWIGEINHSGSTNYNPSLKSRVTISVETSKNQFSLKLSSVTAADTAVYYCARDKWTWYFDLWGRGTLVTVSSASTKGPSVFPLAPSSKSTSGGTAALGCLVKDYFPEPVTVSWNSGALTSGVHTFPAVLQSSGLYSLSSVVTVPSSSLGTQTYICNVNHKPSNTKVDKKVEPKSCDKTHTCPPCPAPELLGGPSVFLFPPKPKDTLMISRTPEVTCVVVDVSHEDPEVKFNWYVDGVEVHNAKTKPREEQYNSTYRVVSVLTVLHQDWLNGKEYKCKVSNKALPAPIEKTISKAKGQPREPQVYTLPPSRDELTKNQVSLTCLVKGFYPSDIAVEWESNGQPENNYKTTPPVLDSDGSFFLYSKLTVDKSRWQQGNVFSCSVMHEALHNHYTQKSLSLSPGK

SEQ ID NO: 4 - protein, 220 aa, Artificial Sequence
  CHAIN: Light chain of U3
DIEMTQSPDSLAVSLGERATINCRSSQSVLYSSSNRNYLAWYQQNPGQPPKLLIYWASTRESGVPDRFSGSGSGTDFTLTISSLQAEDVAVYYCQQYYSTPRTFGQGTKVEIKRTVAAPSVFIFPPSDEQLKSGTASVVCLLNNFYPREAKVQWKVDNALQSGNSQESVTEQDSKDSTYSLSSTLTLSKADYEKHKVYACEVTHQGLSSPVTKSFNRGEC

SEQ ID NO: 5 - protein, 330 aa, Artificial Sequence [sequence omitted]

SEQ ID NO: 6 - protein, 107 aa, Artificial Sequence [sequence omitted]

SEQ ID NO: 7 - protein, 117 aa, Artificial Sequence
  CHAIN: Heavy chain variable region of HER3-29
QVQLVQSGGGLVQPGRSLRLSCAASGFTFDDYAMHWVRQAPGKGLEWVSGISWNSGSIGYADSVKGRFTISRDNAKNSLYLQMNSLRAEDTALYYCAKEGLPGLDYWGQGTLVTVSS

SEQ ID NO: 8 - protein, 108 aa, Artificial Sequence
  CHAIN: Light chain variable region of HER3-29
DIQMTQSPSSLSASIGDRATITCRASQHVGTYLNWYQQKPGKTPKLLISGAANLQSGVPSRFSGSGSGTDFTLTISSLQPEDFATYYCQQSYNTPPFSFGQGTKVEIK

SEQ ID NO: 9 - protein, 7 aa, Artificial Sequence
  DOMAIN: Chothia HCDR1
GFTFDDY

SEQ ID NO: 10 - protein, 6 aa, Artificial Sequence
  DOMAIN: Chothia HCDR2
SWNSGS

SEQ ID NO: 11 - protein, 8 aa, Artificial Sequence
  DOMAIN: Chothia HCDR3
EGLPGLDY

SEQ ID NO: 12 - protein, 11 aa, Artificial Sequence
  DOMAIN: Chothia LCDR1
RASQHVGTYLN

SEQ ID NO: 13 - protein, 7 aa, Artificial Sequence
  DOMAIN: Chothia LCDR2
GAANLQS

SEQ ID NO: 14 - protein, 10 aa, Artificial Sequence
  DOMAIN: Chothia LCDR3
QQSYNTPPFS

SEQ ID NO: 15 - protein, 8 aa, Artificial Sequence
  DOMAIN: IMGT HCDR1
GFTFDDYA

SEQ ID NO: 16 - protein, 8 aa, Artificial Sequence
  DOMAIN: IMGT HCDR2
ISWNSGSI

SEQ ID NO: 17 - protein, 10 aa, Artificial Sequence
  DOMAIN: IMGT HCDR3
AKEGLPGLDY

SEQ ID NO: 18 - protein, 6 aa, Artificial Sequence
  DOMAIN: IMGT LCDR1
QHVGTY

SEQ ID NO: 19 - protein, 3 aa, Artificial Sequence
  DOMAIN: IMGT LCDR2
GAA

SEQ ID NO: 20 - protein, 10 aa, Artificial Sequence
  DOMAIN: IMGT LCDR3
QQSYNTPPFS

SEQ ID NO: 21 - protein, 5 aa, Artificial Sequence
  DOMAIN: Kabat HCDR1
DYAMH

SEQ ID NO: 22 - protein, 17 aa, Artificial Sequence
  DOMAIN: Kabat HCDR2
GISWNSGSIGYADSVKG

SEQ ID NO: 23 - protein, 8 aa, Artificial Sequence
  DOMAIN: Kabat HCDR3
EGLPGLDY

SEQ ID NO: 24 - protein, 11 aa, Artificial Sequence
  DOMAIN: Kabat LCDR1
RASQHVGTYLN

SEQ ID NO: 25 - protein, 7 aa, Artificial Sequence
  DOMAIN: Kabat LCDR2
GAANLQS

SEQ ID NO: 26 - protein, 10 aa, Artificial Sequence
  DOMAIN: Kabat LCDR3
QQSYNTPPFS

SEQ ID NO: 27 - protein, 447 aa, Artificial Sequence
  CHAIN: Heavy chain of HER3-29
QVQLVQSGGGLVQPGRSLRLSCAASGFTFDDYAMHWVRQAPGKGLEWVSGISWNSGSIGYADSVKGRFTISRDNAKNSLYLQMNSLRAEDTALYYCAKEGLPGLDYWGQGTLVTVSSASTKGPSVFPLAPSSKSTSGGTAALGCLVKDYFPEPVTVSWNSGALTSGVHTFPAVLQSSGLYSLSSVVTVPSSSLGTQTYICNVNHKPSNTKVDKKVEPKSCDKTHTCPPCPAPELLGGPSVFLFPPKPKDTLMISRTPEVTCVVVDVSHEDPEVKFNWYVDGVEVHNAKTKPREEQYNSTYRVVSVLTVLHQDWLNGKEYKCKVSNKALPAPIEKTISKAKGQPREPQVYTLPPSRDELTKNQVSLTCLVKGFYPSDIAVEWESNGQPENNYKTTPPVLDSDGSFFLYSKLTVDKSRWQQGNVFSCSVMHEALHNHYTQKSLSLSPGK

SEQ ID NO: 28 - protein, 215 aa, Artificial Sequence
  CHAIN: Light chain of HER3-29
DIQMTQSPSSLSASIGDRATITCRASQHVGTYLNWYQQKPGKTPKLLISGAANLQSGVPSRFSGSGSGTDFTLTISSLQPEDFATYYCQQSYNTPPFSFGQGTKVEIKRTVAAPSVFIFPPSDEQLKSGTASVVCLLNNFYPREAKVQWKVDNALQSGNSQESVTEQDSKDSTYSLSSTLTLSKADYEKHKVYACEVTHQGLSSPVTKSFNRGEC